European Patent Specification EP 3 204 771 B1, published March 12, 2025. Title: METHODS AND SYSTEMS FOR DISTINGUISHING IRRITABLE BOWEL SYNDROME FROM INFLAMMATORY BOWEL DISEASE AND CELIAC DISEASE. Applicant: CEDARS-SINAI MEDICAL CENTER PIMENTEL, Mark CHANG, Christopher. The sequence listing filed with the application follows.

SEQUENCE LISTING (7 sequences)

SEQ ID NO: 1 - protein, 267 aa, Campylobacter coli
MKKIVFLILSFNVLFAALENYNTGTWNLQGSSAATESKWNVSIRQLITGANPMDVLAVQEAGVLPSTAMMTPRQVQPVGVGIPIHEYIWNLGSVSRPSSVYIYYSRVDVGANRVNLAIVSRVQADEVFVLPPPTVASRPIIGIRIGNDAFFNIHALASGGNDAGAIVAAVDMFFRNRPDINWMILGDFNRESGALVTLLDPDLRARTRVVVPPSSTQTSGRTIDYAITGNSNTAALYNPPPIVAILALEGLRTFLASDHFPVNFRRP

SEQ ID NO: 2 - DNA, 804 bp, Campylobacter coli
atgaaaaaaatagtatttttgattttaagttttaatgtattatttgccgctttagaaaattacaacaccggaacttggaatttgcaaggctcatcagctgcaactgaaagcaaatggaatgttagtataagacaactcataaccggtgcaaatcctatggatgttttagctgttcaagaagcgggggttttacctagtacagctatgatgactcctagacaggtacaacccgtgggcgtgggtattcctatacatgaatacatatggaatttaggctctgtatcaagacctagctctgtttatatatattattctagagtggatgtaggagcaaatcgtgtgaatttagctatcgttagcagagtgcaagcggatgaagtttttgttttaccccctccaacagttgcttcaagacctattataggcatacgcataggcaatgatgcttttttcaatatacacgctctagcaagtgggggaaatgacgcaggagccattgtcgctgctgtggatatgttttttagaaatagacctgatattaattggatgattttaggcgattttaatagagaatcaggcgccttagtaaccttgctagatcctgacttaagagcacgcactcgcgtagttgttccgccttcttctacgcaaacaagtggaagaacgattgattatgctatcactggaaattccaacactgcagctttatacaacccaccaccgatagttgcgattttagctttagaaggattaagaacctttttggcttcagatcattttcctgtaaattttagaagaccttag

SEQ ID NO: 3 - protein, 17 aa, Campylobacter jejuni
LDYAITGNSNRQQTYTP

SEQ ID NO: 4 - protein, 18 aa, Campylobacter jejuni
CLDYAITGNSNRQQTYTP

SEQ ID NO: 5 - protein, 265 aa, Campylobacter jejuni
MKKIICLFLSFNLAFANLENFNVGTWNLQGSSAATESKWSVSVRQLVSGANPLDILMIQEAGTLPRTATPTGRHVQQGGTPIDEYEWNLGTLSRPDRVFIYYSRVDVGANRVNLAIVSRMQAEEVIVLPPPTTVSRPIIGIRNGNDAFFNIHALANGGTDVGAIITAVDAHFANMPQVNWMIAGDFNRDPSTITSTVDRELANRIRVVFPTSATQASGGTLDYAITGNSNRQQTYTPPLLAAILMLASLRSHIVSDHFPVNFRKF

SEQ ID NO: 6 - DNA, 51 bp, Campylobacter jejuni
cttgattatgcaattacaggaaattcaaatagacaacaaacctatactcca

SEQ ID NO: 7 - protein, 1066 aa, Homo sapiens
MPVFHTRTIESILEPVAQQISHLVIMHEEGEVDGKAIPDLTAPVAAVQAAVSNLVRVGKETVQTTEDQILKRDMPPAFIKVENACTKLVQAAQMLQSDPYSVPARDYLIDGSRGILSGTSDLLLTFDEAEVRKIIRVCKGILEYLTVAEVVETMEDLVTYTKNLGPGMTKMAKMIDERQQELTHQEHRVMLVNSMNTVKELLPVLISAMKIFVTTKNSKNQGIEEALKNRNFTVEKMSAEINEIIRVLQLTSWDEDAWASKDTEAMKRALASIDSKLNQAKGWLRDPSASPGDAGEQAIRQILDEAGKVGELCAGKERREILGTCKMLGQMTDQVADLRARGQGSSPVAMQKAQQVSQGLDVLTAKVENAARKLEAMTNSKQSIAKKIDAAQNWLADPNGGPEGEEQIRGALAEARKIAELCDDPKERDDILRSLGEISALTSKLADLRRQGKGDSPEARALAKQVATALQNLQTKTNRAVANSRPAKAAVHLEGKIEQAQRWIDNPTVDDRGVGQAAIRGLVAEGHRLANVMMGPYRQDLLAKCDRVDQLTAQLADLAARGEGESPQARALASQLQDSLKDLKARMQEAMTQEVSDVFSDTTTPIKLLAVAATAPPDAPNREEVFDERAANFENHSGKLGATAEKAAAVGTANKSTVEGIQASVKTARELTPQVVSAARILLRNPGNQAAYEHFETMKNQWIDNVEKMTGLVDEAIDTKSLLDASEEAIKKDLDKCKVAMANIQPQMLVAGATSIARRANRILLVAKREVENSEDPKFREAVKAASDELSKTISPMVMDAKAVAGNISDPGLQKSFLDSGYRILGAVAKVREAFQPQEPDFPPPPPDLEQLRLTDELAPPKPPLPEGEVPPPRPPPPEEKDEEFPEQKAGEVINQPMMMAARQLHDEARKWSSKGNDIIAAAKRMALLMAEMSRLVRGGSGTKRALIQCAKDIAKASDEVTRLAKEVAKQCTDKRIRTNLLQVCERIPTISTQLKILSTVKATMLGRTNISDEESEQATEMLVHNAQNLMQSVKETVREAEAASIKIRTDAGFTLRWVRKTPWYQ